European Patent Specification EP 4 036 113 B1, published November 19, 2025. Title: HUMANIZED ANTI-IL17A ANTIBODY AND USE THEREOF. Applicant: SinoCellTech Ltd. The sequence listing filed with the application follows.

SEQUENCE LISTING (43 sequences)

SEQ ID NO: 1 - protein, 155 aa, Artificial Sequence
  Amino acid sequence of Met1-Ala155 of the human IL17A protein (UniProtKB Q16552)
MTPGKTSLVSLLLLLSLEAIVKAGITIPRNPGCPNSEDKNFPRTVMVNLNIHNRNTNTNPKRSSDYYNRSTSPWNLHRNEDPERYPSVIWEAKCRHLGCINADGNVDYHMNSVPIQQEILVLRREPPHCPNSFRLEKILVSVGCTCVTPIVHHVA

SEQ ID NO: 2 - DNA, 54 bp, Artificial Sequence
  Nucleotide sequence of the linker used in the construction of the phage antibody library for the linkage of murine antibody scFv
tctagtggtggcggtggttcgggcggtggtggaggtggtagttctagatcttcc

SEQ ID NO: 3 - DNA, 747 bp, Artificial Sequence
  Nucleotide sequence of murine antibody scFv used in the construction of antibody IL17A-M069
gacattgtgatgtcacagtctccatcctccctggctatgtcagtaggacagaaggtcactatgaactgcaagtccaatcagagccttttaaatagaagcaatcaaaagaactatttggcctggtaccagcagaaaccaggacagtctcctaaacttctggtagactttgcatccactagggaatctggggtccctgatcgcttcataggcagtggatctgggacagatttcagtcttaccatcagcagtgtgcaggctgaggacctggcagattacttctgtcagcaacattataccactccattcacgttcggctcggggaccaagctggaaataaaatctagtggtggcggtggttcgggcggtggtggaggtggtagttctagatcttcccaggcccaccttcaacagtctggggctgagctggtgaggcctggggcttcagtgaagctgtcctgcaaggctttgggctacacatttactgactatgaaatgcactgggtgaaacagacacctgtgcatggcctggaatggattggagttattcatccaggaggtggtggtacggcctacaatcagaagttcaagggcaaggccacactgactgcagacaagtcctccagtacagcctacatggagctcagcagcctgacatctgaggactctgctgtctattactgtacaagaggggatcacgacggaaggactgactactggggccaaggcaccactctcacagtctcctca

SEQ ID NO: 4 - DNA, 354 bp, Artificial Sequence
  Nucleotide sequence of the heavy chain variable region of murine antibody IL17A-M069
caggcccaccttcaacagtctggggctgagctggtgaggcctggggcttcagtgaagctgtcctgcaaggctttgggctacacatttactgactatgaaatgcactgggtgaaacagacacctgtgcatggcctggaatggattggagttattcatccaggaggtggtggtacggcctacaatcagaagttcaagggcaaggccacactgactgcagacaagtcctccagtacagcctacatggagctcagcagcctgacatctgaggactctgctgtctattactgtacaagaggggatcacgacggaaggactgactactggggccaaggcaccactctcacagtctcctca

SEQ ID NO: 5 - DNA, 339 bp, Artificial Sequence
  Nucleotide sequence of the light chain variable region of murine antibody IL17A-M069
gacattgtgatgtcacagtctccatcctccctggctatgtcagtaggacagaaggtcactatgaactgcaagtccaatcagagccttttaaatagaagcaatcaaaagaactatttggcctggtaccagcagaaaccaggacagtctcctaaacttctggtagactttgcatccactagggaatctggggtccctgatcgcttcataggcagtggatctgggacagatttcagtcttaccatcagcagtgtgcaggctgaggacctggcagattacttctgtcagcaacattataccactccattcacgttcggctcggggaccaagctggaaataaaa

SEQ ID NO: 6 - DNA, 975 bp, Artificial Sequence
  Nucleotide sequence of mouse IgG1 heavy chain constant region
gccaaaacgacacccccatctgtctatccactggcccctggatctgctgcccaaactaactccatggtgaccctgggatgcctggtcaagggctatttccctgagccagtgacagtgacctggaactctggatccctgtccagcggtgtgcacaccttcccagctgtcctgcagtctgacctctacactctgagcagctcagtgactgtcccctccagcacctggcccagcgagaccgtcacctgcaacgttgcccacccggccagcagcaccaaggtggacaagaaaattgtgcccagggattgtggttgtaagccttgcatatgtacagtcccagaagtatcatctgtcttcatcttccccccaaagcccaaggatgtgctcaccattactctgactcctaaggtcacgtgtgttgtggtagacatcagcaaggatgatcccgaggtccagttcagctggtttgtagatgatgtggaggtgcacacagctcagacgcaaccccgggaggagcagttcaacagcactttccgctcagtcagtgaacttcccatcatgcaccaggactggctcaatggcaaggagttcaaatgcagggtcaacagtgcagctttccctgcccccatcgagaaaaccatctccaaaaccaaaggcagaccgaaggctccacaggtgtacaccattccacctcccaaggagcagatggccaaggataaagtcagtctgacctgcatgataacagacttcttccctgaagacattactgtggagtggcagtggaatgggcagccagcggagaactacaagaacactcagcccatcatggacacagatggctcttacttcgtctacagcaagctcaatgtgcagaagagcaactgggaggcaggaaatactttcacctgctctgtgttacatgagggcctgcacaaccaccatactgagaagagcctctcccactctcctggtaaataa

SEQ ID NO: 7 - DNA, 325 bp, Artificial Sequence
  Nucleotide sequence of mouse kappa light chain constant region
cgggctgatgctgcaccaactgtatccatcttcccaccatccagtgagcagttaacatctggaggtgcctcagtcgtgtgcttcttgaacaacttctaccccaaagacatcaatgtcaagtggaagattgatggcagtgaacgacaaaatggcgtcctgaacagttggactgatcaggacagcaaagacagcacctacagcatgagcagcaccctcacgttgaccaaggacgagtatgaacgacataacagctatacctgtgaggccactcacaagacatcaacttcacccattgtcaagagcttcaacaggaatgagtgttaaa

SEQ ID NO: 8 - protein, 118 aa, Artificial Sequence
  Amino acid sequence of the heavy chain variable region of murine antibody IL17A-M069
QAHLQQSGAELVRPGASVKLSCKALGYTFTDYEMHWVKQTPVHGLEWIGVIHPGGGGTAYNQKFKGKATLTADKSSSTAYMELSSLTSEDSAVYYCTRGDHDGRTDYWGQGTTLTVSS

SEQ ID NO: 9 - protein, 113 aa, Artificial Sequence
  Amino acid sequence of the light chain variable region of murine antibody IL17A-M069
DIVMSQSPSSLAMSVGQKVTMNCKSNQSLLNRSNQKNYLAWYQQKPGQSPKLLVDFASTRESGVPDRFIGSGSGTDFSLTISSVQAEDLADYFCQQHYTTPFTFGSGTKLEIK

SEQ ID NO: 10 - protein, 14 aa, Artificial Sequence
  Amino acid sequence of the light chain CDR1 of murine antibody IL17A-M069/humanized antibody IL17A-H069
QSLLNRSNQKNYLA

SEQ ID NO: 11 - protein, 7 aa, Artificial Sequence
  Amino acid sequence of the light chain CDR2 of murine antibody IL17A-M069/humanized antibody IL17A-H069
FASTRES

SEQ ID NO: 12 - protein, 9 aa, Artificial Sequence
  Amino acid sequence of the light chain CDR3 of murine antibody IL17A-M069/humanized antibody IL17A-H069
QQHYTTPFT

SEQ ID NO: 13 - protein, 10 aa, Artificial Sequence
  Amino acid sequence of the heavy chain CDR1 of murine antibody IL17A-M069/humanized antibody IL17A-H069
GYTFTDYEMH

SEQ ID NO: 14 - protein, 17 aa, Artificial Sequence
  Amino acid sequence of the heavy chain CDR2 of murine antibody IL17A-M069/humanized antibody IL17A-H069
VIHPGGGGTAYNQKFKG

SEQ ID NO: 15 - protein, 11 aa, Artificial Sequence
  Amino acid sequence of the heavy chain CDR3 of murine antibody IL17A-M069/humanized antibody IL17A-H069
TRGDHDGRTDY

SEQ ID NO: 16 - protein, 447 aa, Artificial Sequence
  Amino acid sequence of the heavy chain of humanized antibody IL17A-H069
EVQLVQSGAEVKKPGATVKISCKASGYTFTDYEMHWVQQAPGHGLEWMGVIHPGGGGTAYNQKFKGRVTITADTSTDTAYMELSSLRSEDTAVYYCTRGDHDGRTDYWGQGTLVTVSSASTKGPSVFPLAPSSKSTSGGTAALGCLVKDYFPEPVTVSWNSGALTSGVHTFPAVLQSSGLYSLSSVVTVPSSSLGTQTYICNVNHKPSNTKVDKKVEPKSCDKTHTCPPCPAPELLGGPSVFLFPPKPKDTLMISRTPEVTCVVVDVSHEDPEVKFNWYVDGVEVHNAKTKPREEQYNSTYRVVSVLTVLHQDWLNGKEYKCKVSNKALPAPIEKTISKAKGQPREPQVYTLPPSRDELTKNQVSLTCLVKGFYPSDIAVEWESNGQPENNYKTTPPVLDSDGSFFLYSKLTVDKSRWQQGNVFSCSVMHEALHNHYTQKSLSLSPG

SEQ ID NO: 17 - protein, 220 aa, Artificial Sequence
  Amino acid sequence of the light chain of humanized antibody IL17A-H069
DIVMTQSPDSLAVSLGERATINCKSSQSLLNRSNQKNYLAWYQQKPGQPPKLLVDFASTRESGVPDRFSGSGSGTDFTLTISSLQAEDVAVYFCQQHYTTPFTFGPGTKVDIKRTVAAPSVFIFPPSDEQLKSGTASVVCLLNNFYPREAKVQWKVDNALQSGNSQESVTEQDSKDSTYSLSSTLTLSKADYEKHKVYACEVTHQGLSSPVTKSFNRGEC

SEQ ID NO: 18 - protein, 466 aa, Artificial Sequence
  Amino acid sequence of the heavy chain of humanized antibody IL17A-H069 containing signal peptide
MELGLSWIFLLAILKGVQCEVQLVQSGAEVKKPGATVKISCKASGYTFTDYEMHWVQQAPGHGLEWMGVIHPGGGGTAYNQKFKGRVTITADTSTDTAYMELSSLRSEDTAVYYCTRGDHDGRTDYWGQGTLVTVSSASTKGPSVFPLAPSSKSTSGGTAALGCLVKDYFPEPVTVSWNSGALTSGVHTFPAVLQSSGLYSLSSVVTVPSSSLGTQTYICNVNHKPSNTKVDKKVEPKSCDKTHTCPPCPAPELLGGPSVFLFPPKPKDTLMISRTPEVTCVVVDVSHEDPEVKFNWYVDGVEVHNAKTKPREEQYNSTYRVVSVLTVLHQDWLNGKEYKCKVSNKALPAPIEKTISKAKGQPREPQVYTLPPSRDELTKNQVSLTCLVKGFYPSDIAVEWESNGQPENNYKTTPPVLDSDGSFFLYSKLTVDKSRWQQGNVFSCSVMHEALHNHYTQKSLSLSPG

SEQ ID NO: 19 - protein, 239 aa, Artificial Sequence
  Amino acid sequence of the light chain of humanized antibody IL17A-H069 containing signal peptide
MGWSCIILFLVATATGVHSDIVMTQSPDSLAVSLGERATINCKSSQSLLNRSNQKNYLAWYQQKPGQPPKLLVDFASTRESGVPDRFSGSGSGTDFTLTISSLQAEDVAVYFCQQHYTTPFTFGPGTKVDIKRTVAAPSVFIFPPSDEQLKSGTASVVCLLNNFYPREAKVQWKVDNALQSGNSQESVTEQDSKDSTYSLSSTLTLSKADYEKHKVYACEVTHQGLSSPVTKSFNRGEC

SEQ ID NO: 20 - protein, 19 aa, Artificial Sequence
  Amino acid sequence of the heavy chain signal peptide of humanized antibody IL17A-H069
MELGLSWIFLLAILKGVQC

SEQ ID NO: 21 - protein, 19 aa, Artificial Sequence
  Amino acid sequence of the light chain signal peptide of humanized antibody IL17A-H069/murine antibody IL17A-M069
MGWSCIILFLVATATGVHS

SEQ ID NO: 22 - protein, 118 aa, Artificial Sequence
  Amino acid sequence of the heavy chain variable region of humanized antibody IL17A-H069
EVQLVQSGAEVKKPGATVKISCKASGYTFTDYEMHWVQQAPGHGLEWMGVIHPGGGGTAYNQKFKGRVTITADTSTDTAYMELSSLRSEDTAVYYCTRGDHDGRTDYWGQGTLVTVSS

SEQ ID NO: 23 - protein, 113 aa, Artificial Sequence
  Amino acid sequence of the light chain variable region of humanized antibody IL17A-H069
DIVMTQSPDSLAVSLGERATINCKSSQSLLNRSNQKNYLAWYQQKPGQPPKLLVDFASTRESGVPDRFSGSGSGTDFTLTISSLQAEDVAVYFCQQHYTTPFTFGPGTKVDIK

SEQ ID NO: 24 - protein, 329 aa, Artificial Sequence
  Amino acid sequence of humanized antibody IL17A-H069 heavy chain constant region
ASTKGPSVFPLAPSSKSTSGGTAALGCLVKDYFPEPVTVSWNSGALTSGVHTFPAVLQSSGLYSLSSVVTVPSSSLGTQTYICNVNHKPSNTKVDKKVEPKSCDKTHTCPPCPAPELLGGPSVFLFPPKPKDTLMISRTPEVTCVVVDVSHEDPEVKFNWYVDGVEVHNAKTKPREEQYNSTYRVVSVLTVLHQDWLNGKEYKCKVSNKALPAPIEKTISKAKGQPREPQVYTLPPSRDELTKNQVSLTCLVKGFYPSDIAVEWESNGQPENNYKTTPPVLDSDGSFFLYSKLTVDKSRWQQGNVFSCSVMHEALHNHYTQKSLSLSPG

SEQ ID NO: 25 - protein, 107 aa, Artificial Sequence [sequence omitted]

SEQ ID NO: 26 - DNA, 1407 bp, Artificial Sequence
  Nucleotide sequence of the humanized antibody IL17A-H069 heavy chain containing signal peptide
atggagttgggactgagctggattttccttttggctattttaaaaggtgtccagtgtgaggtccaacttgtccagtctggagcagaggtgaagaagcctggagccacagtgaagatttcctgtaaggcatctggctacaccttcacagactatgagatgcactgggtccaacaggctcctggccatggattggagtggatgggagtgattcaccctggaggaggaggcacagcctacaaccagaagttcaagggcagggtgaccatcacagcagacaccagcacagacacagcctatatggaactgtcctccctgaggtctgaggacacagcagtctactactgtaccaggggagaccatgatggcaggacagactactggggacaaggcaccctggtgacagtgtcctctgcaagcaccaagggcccatcggtcttccccctggcaccctcctccaagagcacctctgggggcacagcggccctgggctgcctggtcaaggactacttccccgaaccggtgacggtgtcgtggaactcaggcgccctgaccagcggcgtgcacaccttcccggctgtcctacagtcctcaggactctactccctcagcagcgtggtgaccgtgccctccagcagcttgggcacccagacctacatctgcaacgtgaatcacaagcccagcaacaccaaggtggacaagaaagttgagcccaaatcttgtgacaaaactcacacatgcccaccgtgcccagcacctgaactcctggggggaccgtcagtcttcctcttccccccaaaacccaaggacaccctcatgatctcccggacccctgaggtcacgtgcgtggtggtggacgtgagccacgaagaccccgaggtcaagttcaactggtacgtggacggcgtggaggtgcataatgccaagacaaagccgcgggaggagcagtacaacagcacgtaccgtgtggtcagcgtcctcaccgtcctgcaccaggactggctgaatggcaaggagtacaagtgcaaggtctccaacaaagccctcccagcccccatcgagaaaaccatctccaaagccaaagggcagccccgagaaccacaggtgtacaccctgcccccatcccgggatgagctgaccaagaaccaggtcagcctgacctgcctggtcaaaggcttctatcccagcgacatcgccgtggagtgggagagcaatgggcagccggagaacaactacaagaccacgcctcccgtgctggactccgacggctccttcttcctctacagcaagctcaccgtggacaagagcaggtggcagcaggggaacgtcttctcatgctccgtgatgcatgaggctctgcacaaccactacacccagaagtccctgtctctgagccctggctaatagtga

SEQ ID NO: 27 - DNA, 720 bp, Artificial Sequence
  Nucleotide sequence of the humanized antibody IL17A-H069 light chain containing signal peptide
atgggctggtcctgtatcatcctgttcctggtggctacagccacaggagtgcattctgacattgtgatgacccagagccctgactccctggctgtgtccctgggagagagggctaccatcaactgtaagtccagccagtccctgctgaacaggagcaaccagaagaactacctggcttggtatcaacagaagcctggacaacctccaaaactgctggtggactttgccagcaccagggagtctggagtgcctgacaggttctctggctctggctctggcacagacttcaccctgaccatctcctccctccaagcagaggatgtggctgtctacttctgtcaacaacactacaccacaccattcacctttggacctggcaccaaggtggacatcaagcgtacggtggctgcaccatctgtcttcatcttcccgccatctgatgagcagttgaaatctggaactgcctctgttgtgtgcctgctgaataacttctatcccagagaggccaaagtacagtggaaggtggataacgccctccaatcgggtaactcccaggagagtgtcacagagcaggacagcaaggacagcacctacagcctcagcagcaccctgacgctgagcaaagcagactacgagaaacacaaagtctacgcctgcgaagtcacccatcagggcctgagctcgcccgtcacaaagagcttcaacaggggagagtgttaa

SEQ ID NO: 28 - DNA, 57 bp, Artificial Sequence
  Nucleotide sequence of the heavy chain signal peptide of humanized antibody IL17A-H069
atggagttgggactgagctggattttccttttggctattttaaaaggtgtccagtgt

SEQ ID NO: 29 - DNA, 57 bp, Artificial Sequence
  Nucleotide sequence of the light chain signal peptide of humanized antibody IL17A-H069
atgggctggtcctgtatcatcctgttcctggtggctacagccacaggagtgcattct

SEQ ID NO: 30 - DNA, 354 bp, Artificial Sequence
  Nucleotide sequence of the heavy chain variable region of humanized antibody IL17A-H069
gaggtccaacttgtccagtctggagcagaggtgaagaagcctggagccacagtgaagatttcctgtaaggcatctggctacaccttcacagactatgagatgcactgggtccaacaggctcctggccatggattggagtggatgggagtgattcaccctggaggaggaggcacagcctacaaccagaagttcaagggcagggtgaccatcacagcagacaccagcacagacacagcctatatggaactgtcctccctgaggtctgaggacacagcagtctactactgtaccaggggagaccatgatggcaggacagactactggggacaaggcaccctggtgacagtgtcctct

SEQ ID NO: 31 - DNA, 339 bp, Artificial Sequence
  Nucleotide sequence of the light chain variable region of humanized antibody IL17A-H069
gacattgtgatgacccagagccctgactccctggctgtgtccctgggagagagggctaccatcaactgtaagtccagccagtccctgctgaacaggagcaaccagaagaactacctggcttggtatcaacagaagcctggacaacctccaaaactgctggtggactttgccagcaccagggagtctggagtgcctgacaggttctctggctctggctctggcacagacttcaccctgaccatctcctccctccaagcagaggatgtggctgtctacttctgtcaacaacactacaccacaccattcacctttggacctggcaccaaggtggacatcaag

SEQ ID NO: 32 - DNA, 996 bp, Artificial Sequence
  Nucleotide sequence of the heavy chain constant region of humanized antibody IL17A-H069
gcaagcaccaagggcccatcggtcttccccctggcaccctcctccaagagcacctctgggggcacagcggccctgggctgcctggtcaaggactacttccccgaaccggtgacggtgtcgtggaactcaggcgccctgaccagcggcgtgcacaccttcccggctgtcctacagtcctcaggactctactccctcagcagcgtggtgaccgtgccctccagcagcttgggcacccagacctacatctgcaacgtgaatcacaagcccagcaacaccaaggtggacaagaaagttgagcccaaatcttgtgacaaaactcacacatgcccaccgtgcccagcacctgaactcctggggggaccgtcagtcttcctcttccccccaaaacccaaggacaccctcatgatctcccggacccctgaggtcacgtgcgtggtggtggacgtgagccacgaagaccccgaggtcaagttcaactggtacgtggacggcgtggaggtgcataatgccaagacaaagccgcgggaggagcagtacaacagcacgtaccgtgtggtcagcgtcctcaccgtcctgcaccaggactggctgaatggcaaggagtacaagtgcaaggtctccaacaaagccctcccagcccccatcgagaaaaccatctccaaagccaaagggcagccccgagaaccacaggtgtacaccctgcccccatcccgggatgagctgaccaagaaccaggtcagcctgacctgcctggtcaaaggcttctatcccagcgacatcgccgtggagtgggagagcaatgggcagccggagaacaactacaagaccacgcctcccgtgctggactccgacggctccttcttcctctacagcaagctcaccgtggacaagagcaggtggcagcaggggaacgtcttctcatgctccgtgatgcatgaggctctgcacaaccactacacccagaagtccctgtctctgagccctggctaatagtga

SEQ ID NO: 33 - DNA, 324 bp, Artificial Sequence
  Nucleotide sequence of the light chain constant region of humanized antibody IL17A-H069
cgtacggtggctgcaccatctgtcttcatcttcccgccatctgatgagcagttgaaatctggaactgcctctgttgtgtgcctgctgaataacttctatcccagagaggccaaagtacagtggaaggtggataacgccctccaatcgggtaactcccaggagagtgtcacagagcaggacagcaaggacagcacctacagcctcagcagcaccctgacgctgagcaaagcagactacgagaaacacaaagtctacgcctgcgaagtcacccatcagggcctgagctcgcccgtcacaaagagcttcaacaggggagagtgttaa

SEQ ID NO: 34 - protein, 249 aa, Artificial Sequence
  Amino acid sequence of murine antibody scFv used in the construction of antibody IL17A-M069
DIVMSQSPSSLAMSVGQKVTMNCKSNQSLLNRSNQKNYLAWYQQKPGQSPKLLVDFASTRESGVPDRFIGSGSGTDFSLTISSVQAEDLADYFCQQHYTTPFTFGSGTKLEIKSSGGGGSGGGGGGSSRSSQAHLQQSGAELVRPGASVKLSCKALGYTFTDYEMHWVKQTPVHGLEWIGVIHPGGGGTAYNQKFKGKATLTADKSSSTAYMELSSLTSEDSAVYYCTRGDHDGRTDYWGQGTTLTVSS

SEQ ID NO: 35 - protein, 18 aa, Artificial Sequence
  Amino acid sequence of the linker used in the construction of the phage antibody library for the linkage of murine antibody scFv
SSGGGGSGGGGGGSSRSS

SEQ ID NO: 36 - DNA, 1386 bp, Artificial Sequence
  Nucleotide sequence of the murine antibody IL17A-M069 heavy chain containing signal peptide
atgggctggtccctgattctgctgttcctggtggctgtggctaccagggtgctgagccaggcccaccttcaacagtctggggctgagctggtgaggcctggggcttcagtgaagctgtcctgcaaggctttgggctacacatttactgactatgaaatgcactgggtgaaacagacacctgtgcatggcctggaatggattggagttattcatccaggaggtggtggtacggcctacaatcagaagttcaagggcaaggccacactgactgcagacaagtcctccagtacagcctacatggagctcagcagcctgacatctgaggactctgctgtctattactgtacaagaggggatcacgacggaaggactgactactggggccaaggcaccactctcacagtctcctcagccaaaacgacacccccatctgtctatccactggcccctggatctgctgcccaaactaactccatggtgaccctgggatgcctggtcaagggctatttccctgagccagtgacagtgacctggaactctggatccctgtccagcggtgtgcacaccttcccagctgtcctgcagtctgacctctacactctgagcagctcagtgactgtcccctccagcacctggcccagcgagaccgtcacctgcaacgttgcccacccggccagcagcaccaaggtggacaagaaaattgtgcccagggattgtggttgtaagccttgcatatgtacagtcccagaagtatcatctgtcttcatcttccccccaaagcccaaggatgtgctcaccattactctgactcctaaggtcacgtgtgttgtggtagacatcagcaaggatgatcccgaggtccagttcagctggtttgtagatgatgtggaggtgcacacagctcagacgcaaccccgggaggagcagttcaacagcactttccgctcagtcagtgaacttcccatcatgcaccaggactggctcaatggcaaggagttcaaatgcagggtcaacagtgcagctttccctgcccccatcgagaaaaccatctccaaaaccaaaggcagaccgaaggctccacaggtgtacaccattccacctcccaaggagcagatggccaaggataaagtcagtctgacctgcatgataacagacttcttccctgaagacattactgtggagtggcagtggaatgggcagccagcggagaactacaagaacactcagcccatcatggacacagatggctcttacttcgtctacagcaagctcaatgtgcagaagagcaactgggaggcaggaaatactttcacctgctctgtgttacatgagggcctgcacaaccaccatactgagaagagcctctcccactctcctggtaaataa

SEQ ID NO: 37 - DNA, 721 bp, Artificial Sequence
  Nucleotide sequence of the murine antibody IL17A-M069 light chain containing signal peptide
atgggctggtcctgtatcatcctgttcctggtggctacagccacaggagtgcatagcgacattgtgatgtcacagtctccatcctccctggctatgtcagtaggacagaaggtcactatgaactgcaagtccaatcagagccttttaaatagaagcaatcaaaagaactatttggcctggtaccagcagaaaccaggacagtctcctaaacttctggtagactttgcatccactagggaatctggggtccctgatcgcttcataggcagtggatctgggacagatttcagtcttaccatcagcagtgtgcaggctgaggacctggcagattacttctgtcagcaacattataccactccattcacgttcggctcggggaccaagctggaaataaaacgggctgatgctgcaccaactgtatccatcttcccaccatccagtgagcagttaacatctggaggtgcctcagtcgtgtgcttcttgaacaacttctaccccaaagacatcaatgtcaagtggaagattgatggcagtgaacgacaaaatggcgtcctgaacagttggactgatcaggacagcaaagacagcacctacagcatgagcagcaccctcacgttgaccaaggacgagtatgaacgacataacagctatacctgtgaggccactcacaagacatcaacttcacccattgtcaagagcttcaacaggaatgagtgttaaa

SEQ ID NO: 38 - protein, 461 aa, Artificial Sequence
  Amino acid sequence of the heavy chain of murine antibody IL17A-M069 containing signal peptide
MGWSLILLFLVAVATRVLSQAHLQQSGAELVRPGASVKLSCKALGYTFTDYEMHWVKQTPVHGLEWIGVIHPGGGGTAYNQKFKGKATLTADKSSSTAYMELSSLTSEDSAVYYCTRGDHDGRTDYWGQGTTLTVSSAKTTPPSVYPLAPGSAAQTNSMVTLGCLVKGYFPEPVTVTWNSGSLSSGVHTFPAVLQSDLYTLSSSVTVPSSTWPSETVTCNVAHPASSTKVDKKIVPRDCGCKPCICTVPEVSSVFIFPPKPKDVLTITLTPKVTCVVVDISKDDPEVQFSWFVDDVEVHTAQTQPREEQFNSTFRSVSELPIMHQDWLNGKEFKCRVNSAAFPAPIEKTISKTKGRPKAPQVYTIPPPKEQMAKDKVSLTCMITDFFPEDITVEWQWNGQPAENYKNTQPIMDTDGSYFVYSKLNVQKSNWEAGNTFTCSVLHEGLHNHHTEKSLSHSPGK

SEQ ID NO: 39 - protein, 239 aa, Artificial Sequence
  Amino acid sequence of the light chain of murine antibody IL17A-M069 containing signal peptide
MGWSCIILFLVATATGVHSDIVMSQSPSSLAMSVGQKVTMNCKSNQSLLNRSNQKNYLAWYQQKPGQSPKLLVDFASTRESGVPDRFIGSGSGTDFSLTISSVQAEDLADYFCQQHYTTPFTFGSGTKLEIKRADAAPTVSIFPPSSEQLTSGGASVVCFLNNFYPKDINVKWKIDGSERQNGVLNSWTDQDSKDSTYSMSSTLTLTKDEYERHNSYTCEATHKTSTSPIVKSFNRNEC

SEQ ID NO: 40 - protein, 324 aa, Artificial Sequence
  Amino acid sequence of the heavy chain constant region of murine antibody IL17A-M069
AKTTPPSVYPLAPGSAAQTNSMVTLGCLVKGYFPEPVTVTWNSGSLSSGVHTFPAVLQSDLYTLSSSVTVPSSTWPSETVTCNVAHPASSTKVDKKIVPRDCGCKPCICTVPEVSSVFIFPPKPKDVLTITLTPKVTCVVVDISKDDPEVQFSWFVDDVEVHTAQTQPREEQFNSTFRSVSELPIMHQDWLNGKEFKCRVNSAAFPAPIEKTISKTKGRPKAPQVYTIPPPKEQMAKDKVSLTCMITDFFPEDITVEWQWNGQPAENYKNTQPIMDTDGSYFVYSKLNVQKSNWEAGNTFTCSVLHEGLHNHHTEKSLSHSPGK

SEQ ID NO: 41 - protein, 107 aa, Artificial Sequence
  Amino acid sequence of the light chain constant region of murine antibody IL17A-M069
RADAAPTVSIFPPSSEQLTSGGASVVCFLNNFYPKDINVKWKIDGSERQNGVLNSWTDQDSKDSTYSMSSTLTLTKDEYERHNSYTCEATHKTSTSPIVKSFNRNEC

SEQ ID NO: 42 - protein, 19 aa, Artificial Sequence
  Amino acid sequence of the heavy chain signal peptide of murine antibody IL17A-M069
MGWSLILLFLVAVATRVLS

SEQ ID NO: 43 - DNA, 57 bp, Artificial Sequence
  Nucleotide sequence of the heavy chain signal peptide of murine antibody IL17A-M069
atgggctggtccctgattctgctgttcctggtggctgtggctaccagggtgctgagc